European Patent Application EP 4 484 446 A1, published January 1, 2025. Title: Antibody, drug conjugate and use thereof. Applicant: EVOPOINT BIOSCIENCES CO., LTD. The sequence listing filed with the application follows.

SEQUENCE LISTING (108 sequences)

SEQ ID NO: 1 - protein, 118 aa, artificial sequence
EVQLVESGGGLVQPGGSLRLSCAASGFAFSDSGMHWVRQAPGKGLEWVAYISRDSNTIYYADSVKGRFTISRDNAKNSLYLQMNSLRAEDTAVYYCGRRYYGDYFDYWGQGTLVTVSS

SEQ ID NO: 2 - protein, 107 aa, artificial sequence
DIVLTQSPATLSLSPGERATLSCRASQRVTNYLHWYQQKPGQSPRLLIKYASQSISGIPARFSGSGSGTDFTLTISSLEPEDFAVYFCQQSYNWPLTFGQGTKVEIK

SEQ ID NO: 3 - protein, 118 aa, artificial sequence
EVQLVESGGGLVKPGGSLRLSCAASGFTFSDYGMFWVRQAPGKGLEWVAYISRGSTTIYYADSVKGRFTISRDNAKNSLYLQMNSLRAEDTAVYFCTRRYYGDYFDYWGQGTLVTVSS

SEQ ID NO: 4 - protein, 107 aa, artificial sequence
EIVLTQSPDFQSVTPKEKVTITCRASQSISNYLHWYQQKPDQSPKLLIKYASQSISGVPSRFSGSGSGTDFTLTINSLEAEDAATYFCQQSYNWPLTFGQGTKVEIK

SEQ ID NO: 5 - protein, 118 aa, artificial sequence
QVQLVQSGAEVKQPGASVKVSCKASGYTFTTYWMHWVRQAPGQGLEWMGMIDPSDSYTTYAQKFQGRVTLTVDTSTSTAYMELSSLRSEDTAVYYCARGSGPGLFAYWGQGTLVTVSS

SEQ ID NO: 6 - protein, 107 aa, artificial sequence
DIQETQSPSSLSASVGDRVTITCRASQDIRNYLNWYQQKPGKAPKLLIYHTSRLQSGVPSRFSGSGSGTDYTLTISSLQPEDFATYYCQQGNMPPYTFGQGTKVEIK

SEQ ID NO: 7 - protein, 118 aa, artificial sequence
QVQLVQSGAEVKKPGASVKVSCKASGYTFTTYWMHWVRQAPGQGLEWMGMIDPSDSYTSYAQKFQGRVTLTVDTSTSTAYMELSSLRSEDTAVYYCTRGSGPGLFAYWGQGTLVTVSS

SEQ ID NO: 8 - protein, 107 aa, artificial sequence
DIQETQSPSSLSASVGDRVTITCRASQGISNYLNWYQQKPGKAPKLLIYHTSRLHSGVPSRFSGSVSGTDFTLTISSLQPEDFATYFCQQGNTLPYTFGQGTKVEIK

SEQ ID NO: 9 - protein, 7 aa, artificial sequence
GFAFSDS

SEQ ID NO: 10 - protein, 6 aa, artificial sequence
SRDSNT

SEQ ID NO: 11 - protein, 9 aa, artificial sequence
RYYGDYFDY

SEQ ID NO: 12 - protein, 10 aa, artificial sequence
GFAFSDSGMH

SEQ ID NO: 13 - protein, 10 aa, artificial sequence
YISRDSNTIY

SEQ ID NO: 14 - protein, 9 aa, artificial sequence
RYYGDYFDY

SEQ ID NO: 15 - protein, 5 aa, artificial sequence
DSGMH

SEQ ID NO: 16 - protein, 17 aa, artificial sequence
YISRDSNTIYYADSVKG

SEQ ID NO: 17 - protein, 9 aa, artificial sequence
RYYGDYFDY

SEQ ID NO: 18 - protein, 8 aa, artificial sequence
GFAFSDSG

SEQ ID NO: 19 - protein, 8 aa, artificial sequence
ISRDSNTI

SEQ ID NO: 20 - protein, 11 aa, artificial sequence
GRRYYGDYFDY

SEQ ID NO: 21 - protein, 11 aa, artificial sequence
RASQRVTNYLH

SEQ ID NO: 22 - protein, 7 aa, artificial sequence
YASQSIS

SEQ ID NO: 23 - protein, 9 aa, artificial sequence
QQSYNWPLT

SEQ ID NO: 24 - protein, 11 aa, artificial sequence
RASQRVTNYLH

SEQ ID NO: 25 - protein, 7 aa, artificial sequence
YASQSIS

SEQ ID NO: 26 - protein, 9 aa, artificial sequence
QQSYNWPLT

SEQ ID NO: 27 - protein, 11 aa, artificial sequence
RASQRVTNYLH

SEQ ID NO: 28 - protein, 7 aa, artificial sequence
YASQSIS

SEQ ID NO: 29 - protein, 9 aa, artificial sequence
QQSYNWPLT

SEQ ID NO: 30 - protein, 6 aa, artificial sequence
QRVTNY

SEQ ID NO: 31 - skipped

SEQ ID NO: 32 - protein, 9 aa, artificial sequence
QQSYNWPLT

SEQ ID NO: 33 - protein, 7 aa, artificial sequence
GFTFSDY

SEQ ID NO: 34 - protein, 6 aa, artificial sequence
SRGSTT

SEQ ID NO: 35 - protein, 9 aa, artificial sequence
RYYGDYFDY

SEQ ID NO: 36 - protein, 10 aa, artificial sequence
GFTFSDYGMF

SEQ ID NO: 37 - protein, 10 aa, artificial sequence
YISRGSTTIY

SEQ ID NO: 38 - protein, 9 aa, artificial sequence
RYYGDYFDY

SEQ ID NO: 39 - protein, 5 aa, artificial sequence
DYGMF

SEQ ID NO: 40 - protein, 17 aa, artificial sequence
YISRGSTTIYYADSVKG

SEQ ID NO: 41 - protein, 9 aa, artificial sequence
RYYGDYFDY

SEQ ID NO: 42 - protein, 8 aa, artificial sequence
GFTFSDYG

SEQ ID NO: 43 - protein, 8 aa, artificial sequence
ISRGSTTI

SEQ ID NO: 44 - protein, 11 aa, artificial sequence
TRRYYGDYFDY

SEQ ID NO: 45 - protein, 11 aa, artificial sequence
RASQSISNYLH

SEQ ID NO: 46 - protein, 7 aa, artificial sequence
YASQSIS

SEQ ID NO: 47 - protein, 9 aa, artificial sequence
QQSYNWPLT

SEQ ID NO: 48 - protein, 11 aa, artificial sequence
RASQSISNYLH

SEQ ID NO: 49 - protein, 7 aa, artificial sequence
YASQSIS

SEQ ID NO: 50 - protein, 9 aa, artificial sequence
QQSYNWPLT

SEQ ID NO: 51 - protein, 11 aa, artificial sequence
RASQSISNYLH

SEQ ID NO: 52 - protein, 7 aa, artificial sequence
YASQSIS

SEQ ID NO: 53 - protein, 9 aa, artificial sequence
QQSYNWPLT

SEQ ID NO: 54 - protein, 6 aa, artificial sequence
QSISNY

SEQ ID NO: 55 - skipped

SEQ ID NO: 56 - protein, 9 aa, artificial sequence
QQSYNWPLT

SEQ ID NO: 57 - protein, 7 aa, artificial sequence
GYTFTTY

SEQ ID NO: 58 - protein, 6 aa, artificial sequence
DPSDSY

SEQ ID NO: 59 - protein, 9 aa, artificial sequence
GSGPGLFAY

SEQ ID NO: 60 - protein, 10 aa, artificial sequence
GYTFTTYWMH

SEQ ID NO: 61 - protein, 10 aa, artificial sequence
MIDPSDSYTT

SEQ ID NO: 62 - protein, 9 aa, artificial sequence
GSGPGLFAY

SEQ ID NO: 63 - protein, 5 aa, artificial sequence
TYWMH

SEQ ID NO: 64 - protein, 17 aa, artificial sequence
MIDPSDSYTTYAQKFQG

SEQ ID NO: 65 - protein, 9 aa, artificial sequence
GSGPGLFAY

SEQ ID NO: 66 - protein, 8 aa, artificial sequence
GYTFTTYW

SEQ ID NO: 67 - protein, 8 aa, artificial sequence
IDPSDSYT

SEQ ID NO: 68 - protein, 11 aa, artificial sequence
ARGSGPGLFAY

SEQ ID NO: 69 - protein, 11 aa, artificial sequence
RASQDIRNYLN

SEQ ID NO: 70 - protein, 7 aa, artificial sequence
HTSRLQS

SEQ ID NO: 71 - protein, 9 aa, artificial sequence
QQGNMPPYT

SEQ ID NO: 72 - protein, 11 aa, artificial sequence
RASQDIRNYLN

SEQ ID NO: 73 - protein, 7 aa, artificial sequence
HTSRLQS

SEQ ID NO: 74 - protein, 9 aa, artificial sequence
QQGNMPPYT

SEQ ID NO: 75 - protein, 11 aa, artificial sequence
RASQDIRNYLN

SEQ ID NO: 76 - protein, 7 aa, artificial sequence
HTSRLQS

SEQ ID NO: 77 - protein, 9 aa, artificial sequence
QQGNMPPYT

SEQ ID NO: 78 - protein, 6 aa, artificial sequence
QDIRNY

SEQ ID NO: 79 - skipped

SEQ ID NO: 80 - protein, 9 aa, artificial sequence
QQGNMPPYT

SEQ ID NO: 81 - protein, 7 aa, artificial sequence
GYTFTTY

SEQ ID NO: 82 - protein, 6 aa, artificial sequence
DPSDSY

SEQ ID NO: 83 - protein, 9 aa, artificial sequence
GSGPGLFAY

SEQ ID NO: 84 - protein, 10 aa, artificial sequence
GYTFTTYWMH

SEQ ID NO: 85 - protein, 10 aa, artificial sequence
MIDPSDSYTS

SEQ ID NO: 86 - protein, 9 aa, artificial sequence
GSGPGLFAY

SEQ ID NO: 87 - protein, 5 aa, artificial sequence
TYWMH

SEQ ID NO: 88 - protein, 17 aa, artificial sequence
MIDPSDSYTSYAQKFQG

SEQ ID NO: 89 - protein, 9 aa, artificial sequence
GSGPGLFAY

SEQ ID NO: 90 - protein, 8 aa, artificial sequence
GYTFTTYW

SEQ ID NO: 91 - protein, 8 aa, artificial sequence
IDPSDSYT

SEQ ID NO: 92 - protein, 11 aa, artificial sequence
TRGSGPGLFAY

SEQ ID NO: 93 - protein, 11 aa, artificial sequence
RASQGISNYLN

SEQ ID NO: 94 - protein, 7 aa, artificial sequence
HTSRLHS

SEQ ID NO: 95 - protein, 9 aa, artificial sequence
QQGNTLPYT

SEQ ID NO: 96 - protein, 11 aa, artificial sequence
RASQGISNYLN

SEQ ID NO: 97 - protein, 7 aa, artificial sequence
HTSRLHS

SEQ ID NO: 98 - protein, 9 aa, artificial sequence
QQGNTLPYT

SEQ ID NO: 99 - protein, 11 aa, artificial sequence
RASQGISNYLN

SEQ ID NO: 100 - protein, 7 aa, artificial sequence
HTSRLHS

SEQ ID NO: 101 - protein, 9 aa, artificial sequence
QQGNTLPYT

SEQ ID NO: 102 - protein, 6 aa, artificial sequence
QGISNY

SEQ ID NO: 103 - skipped

SEQ ID NO: 104 - protein, 9 aa, artificial sequence
QQGNTLPYT

SEQ ID NO: 105 - protein, 107 aa, artificial sequence [sequence omitted]

SEQ ID NO: 106 - protein, 330 aa, artificial sequence [sequence omitted]

SEQ ID NO: 107 - protein, 118 aa, artificial sequence
EVQLLESGGGLVQPGGSLRLSCAASGFTFSNYAMSWVRQAPGKGLEWVSSISGSGDYTYYTDSVKGRFTISRDNSKNTLYLQMNSLRAEDTAVYYCARSPWGYYLDSWGQGTLVTVSS

SEQ ID NO: 108 - protein, 107 aa, artificial sequence
EIVLTQSPGTLSLSPGERATLSCRASQSVSSSYLAWYQQKPGQAPRLLIYGASSRATGIPDRFSGSGSGTDFTLTISRLEPEDFAVYYCQQYGSSLTFGGGTKVEIK